European Patent Application EP 4 703 469 A1, published March 4, 2026. Title: Fusion proteins, methods and compositions for efficient serine integrase-mediated gene transfer in human cells. Applicant: Charité - Universitätsmedizin Berlin Körperschaft des öffentlichen Rechts. Application EP. The sequence listing filed with the application follows.

SEQUENCE LISTING (74 sequences)

SEQ ID NO: 1 - protein, 526 aa, unidentified
MGPSAFSYVRFSSGKQAKGSSEHRQRAMLGQWLEQHPSFTLSDLRFEDLGRSGFSGEHLDHGLGQLLAAIDSGAIKSGDVILVEAVDRIGRLEPLEMLPLFSRIVKAGVSVITLEDGHVYDRSSVNETSLFLLVAKIQQAHEYSNRLSRRINASYTARREKAKAGLGIKRETPVWLTTDGQLVPHVAPHIAQAFQDYADGLGERRICRKLRESGLEEFSKTNATTVRRWLKNRTAIGYWNDIPDVYPHVVDPALFYQVQQRLDAPKVDRAKPSAHYLTGLVKCAVCGRNYNYKQRKHTDPAMLCTSRARLAGEGCSNSKTYPVIVLDQVRKLTSLPFLQHAMESASSQADPSSQRLAVIDGEIGELSRKISEATKALLVLGFTPEIQESLEQLKTAREALEEERATLLLPQAEKLTTAQLEAFSNGLLDDEPMKLNHVLQTAGYSMVVHPDGSIDVDGKRFVYEGASRKEKVYKLRLIGEDKQWSLPILTPQMATYKSLFMAAVRLPGDPSEEELRRFEEAKHSER

SEQ ID NO: 2 - protein, 7 aa, simian virus 40
PKKKRKV

SEQ ID NO: 3 - protein, 11 aa, Homo sapiens
DYPAAKRVKLD

SEQ ID NO: 4 - protein, 9 aa, Homo sapiens
PAAKRVKLD

SEQ ID NO: 5 - protein, 16 aa, Homo sapiens
KRPAATKKAGQAKKKK

SEQ ID NO: 6 - protein, 21 aa, Homo sapiens
GKRKLITSEEERSPAKRGRKS

SEQ ID NO: 7 - protein, 22 aa, Homo sapiens
KGKKGRTQKEKKAARARSKGKN

SEQ ID NO: 8 - protein, 28 aa, Homo sapiens
RKRCAAGVGGGPAGCPAPGSTPLKKPRR

SEQ ID NO: 9 - protein, 36 aa, Homo sapiens
RKPVTAQERQREREEKRRRRQERAKEREKRRQERER

SEQ ID NO: 10 - protein, 27 aa, Homo sapiens
FGNYNNQSSNFGPMKGGNFGGRSSGPY

SEQ ID NO: 11 - protein, 27 aa, Homo sapiens
TLLLRETMNNLGVSDHAVLSRKTPQPY

SEQ ID NO: 12 - protein, 11 aa, Homo sapiens
KRTADGSEFES

SEQ ID NO: 13 - protein, 11 aa, Homo sapiens
YRPRPKRTCVI

SEQ ID NO: 14 - protein, 24 aa, Homo sapiens
SRRRKANPTKLSENAKKLAKEVEN

SEQ ID NO: 15 - protein, 34 aa, synthetic construct
KRPAATKKAGQAKKKKGSKRPAATKKAGQAKKKK

SEQ ID NO: 16 - protein, 533 aa, synthetic construct
MGPSAFSYVRFSSGKQAKGSSEHRQRAMLGQWLEQHPSFTLSDLRFEDLGRSGFSGEHLDHGLGQLLAAIDSGAIKSGDVILVEAVDRIGRLEPLEMLPLFSRIVKAGVSVITLEDGHVYDRSSVNETSLFLLVAKIQQAHEYSNRLSRRINASYTARREKAKAGLGIKRETPVWLTTDGQLVPHVAPHIAQAFQDYADGLGERRICRKLRESGLEEFSKTNATTVRRWLKNRTAIGYWNDIPDVYPHVVDPALFYQVQQRLDAPKVDRAKPSAHYLTGLVKCAVCGRNYNYKQRKHTDPAMLCTSRARLAGEGCSNSKTYPVIVLDQVRKLTSLPFLQHAMESASSQADPSSQRLAVIDGEIGELSRKISEATKALLVLGFTPEIQESLEQLKTAREALEEERATLLLPQAEKLTTAQLEAFSNGLLDDEPMKLNHVLQTAGYSMVVHPDGSIDVDGKRFVYEGASRKEKVYKLRLIGEDKQWSLPILTPQMATYKSLFMAAVRLPGDPSEEELRRFEEAKHSERPKKKRKV

SEQ ID NO: 17 - DNA, 1599 bp, synthetic construct
  source 1..1599: mol_type = other DNA
atgggccctagcgccttcagctacgtgcgctttagcagcggcaagcaggccaagggcagctctgaacacagacagagagccatgctgggacagtggctggaacagcaccctagcttcacactgagtgatctgcggttcgaggacctgggcagaagcggattcagcggcgagcacctggatcacggcctgggccagctgctggctgctatcgacagcggcgccatcaagagcggagatgtgatcctggtcgaggccgtggacagaatcggcagactggagcctctggaaatgctgcctctgttctccagaatcgtgaaggccggcgtgtccgttatcaccctggaagatggccacgtttacgaccggagctccgtgaacgagacatctctgtttctgctggtggccaaaatccagcaggcccacgagtactctaatagactgtctcgaagaatcaacgcctcttacaccgctcggagagaaaaagctaaagcaggcctgggcatcaagagagagacacctgtgtggctgaccacagacggccaactggtgcctcacgtggcccctcacatcgcccaggcttttcaggactacgccgatggcctgggagagagaaggatttgtagaaagctgcgggagagcggcctggaagaattctccaagaccaacgccaccaccgtgcggagatggctgaagaaccggaccgccattggatattggaacgacatccctgatgtgtaccctcatgtcgtggaccctgctctgttctaccaggtgcagcagcgcctggacgcccctaaggtggacagagccaagcccagcgctcactacctgacaggcctcgtgaagtgcgccgtgtgcggcagaaactacaactacaaacagcggaagcacaccgaccccgctatgctgtgcaccagcagagccagactggccggggaaggctgcagcaatagcaagacataccccgtgatagttctggaccaggtgcggaagctgaccagcctgccgttcctgcaacacgccatggaatccgcctcatctcaggccgacccaagcagccagagactggccgtgatcgacggcgaaatcggcgagctgtccagaaagatcagcgaggccacaaaggccctgctggtgctgggcttcacccctgagatccaggagagcctggaacagctcaagaccgccagagaagccctggaggaagaaagagccaccctgctgctgcctcaggccgagaagctgacaacagctcagctggaggccttcagcaacggcctgctggacgacgagcccatgaagctcaaccacgtgcttcagaccgccggctacagcatggtggtgcaccccgacggctctatcgacgtggatggaaaaagattcgtgtacgagggcgctagccggaaagagaaagtgtacaagctgagactgatcggcgaggataagcagtggagcctgcccatcctgaccccacagatggccacttacaagtccctgttcatggccgctgtgcggctgcctggcgaccccagcgaggaagagctgagacggttcgaggaagccaagcacagcgagcggcccaagaagaagaggaaagtc

SEQ ID NO: 18 - protein, 535 aa, synthetic construct
MGPSAFSYVRFSSGKQAKGSSEHRQRAMLGQWLEQHPSFTLSDLRFEDLGRSGFSGEHLDHGLGQLLAAIDSGAIKSGDVILVEAVDRIGRLEPLEMLPLFSRIVKAGVSVITLEDGHVYDRSSVNETSLFLLVAKIQQAHEYSNRLSRRINASYTARREKAKAGLGIKRETPVWLTTDGQLVPHVAPHIAQAFQDYADGLGERRICRKLRESGLEEFSKTNATTVRRWLKNRTAIGYWNDIPDVYPHVVDPALFYQVQQRLDAPKVDRAKPSAHYLTGLVKCAVCGRNYNYKQRKHTDPAMLCTSRARLAGEGCSNSKTYPVIVLDQVRKLTSLPFLQHAMESASSQADPSSQRLAVIDGEIGELSRKISEATKALLVLGFTPEIQESLEQLKTAREALEEERATLLLPQAEKLTTAQLEAFSNGLLDDEPMKLNHVLQTAGYSMVVHPDGSIDVDGKRFVYEGASRKEKVYKLRLIGEDKQWSLPILTPQMATYKSLFMAAVRLPGDPSEEELRRFEEAKHSERPAAKRVKLD

SEQ ID NO: 19 - DNA, 1605 bp, synthetic construct
  source 1..1605: mol_type = other DNA
atgggccctagcgccttcagctacgtgcgctttagcagcggcaagcaggccaagggcagctctgaacacagacagagagccatgctgggacagtggctggaacagcaccctagcttcacactgagtgatctgcggttcgaggacctgggcagaagcggattcagcggcgagcacctggatcacggcctgggccagctgctggctgctatcgacagcggcgccatcaagagcggagatgtgatcctggtcgaggccgtggacagaatcggcagactggagcctctggaaatgctgcctctgttctccagaatcgtgaaggccggcgtgtccgttatcaccctggaagatggccacgtttacgaccggagctccgtgaacgagacatctctgtttctgctggtggccaaaatccagcaggcccacgagtactctaatagactgtctcgaagaatcaacgcctcttacaccgctcggagagaaaaagctaaagcaggcctgggcatcaagagagagacacctgtgtggctgaccacagacggccaactggtgcctcacgtggcccctcacatcgcccaggcttttcaggactacgccgatggcctgggagagagaaggatttgtagaaagctgcgggagagcggcctggaagaattctccaagaccaacgccaccaccgtgcggagatggctgaagaaccggaccgccattggatattggaacgacatccctgatgtgtaccctcatgtcgtggaccctgctctgttctaccaggtgcagcagcgcctggacgcccctaaggtggacagagccaagcccagcgctcactacctgacaggcctcgtgaagtgcgccgtgtgcggcagaaactacaactacaaacagcggaagcacaccgaccccgctatgctgtgcaccagcagagccagactggccggggaaggctgcagcaatagcaagacataccccgtgatagttctggaccaggtgcggaagctgaccagcctgccgttcctgcaacacgccatggaatccgcctcatctcaggccgacccaagcagccagagactggccgtgatcgacggcgaaatcggcgagctgtccagaaagatcagcgaggccacaaaggccctgctggtgctgggcttcacccctgagatccaggagagcctggaacagctcaagaccgccagagaagccctggaggaagaaagagccaccctgctgctgcctcaggccgagaagctgacaacagctcagctggaggccttcagcaacggcctgctggacgacgagcccatgaagctcaaccacgtgcttcagaccgccggctacagcatggtggtgcaccccgacggctctatcgacgtggatggaaaaagattcgtgtacgagggcgctagccggaaagagaaagtgtacaagctgagactgatcggcgaggataagcagtggagcctgcccatcctgaccccacagatggccacttacaagtccctgttcatggccgctgtgcggctgcctggcgaccccagcgaggaagagctgagacggttcgaggaagccaagcacagcgagcggcctgctgctaagagagtgaaactggat

SEQ ID NO: 20 - protein, 550 aa, synthetic construct
MGPSAFSYVRFSSGKQAKGSSEHRQRAMLGQWLEQHPSFTLSDLRFEDLGRSGFSGEHLDHGLGQLLAAIDSGAIKSGDVILVEAVDRIGRLEPLEMLPLFSRIVKAGVSVITLEDGHVYDRSSVNETSLFLLVAKIQQAHEYSNRLSRRINASYTARREKAKAGLGIKRETPVWLTTDGQLVPHVAPHIAQAFQDYADGLGERRICRKLRESGLEEFSKTNATTVRRWLKNRTAIGYWNDIPDVYPHVVDPALFYQVQQRLDAPKVDRAKPSAHYLTGLVKCAVCGRNYNYKQRKHTDPAMLCTSRARLAGEGCSNSKTYPVIVLDQVRKLTSLPFLQHAMESASSQADPSSQRLAVIDGEIGELSRKISEATKALLVLGFTPEIQESLEQLKTAREALEEERATLLLPQAEKLTTAQLEAFSNGLLDDEPMKLNHVLQTAGYSMVVHPDGSIDVDGKRFVYEGASRKEKVYKLRLIGEDKQWSLPILTPQMATYKSLFMAAVRLPGDPSEEELRRFEEAKHSERSRRRKANPTKLSENAKKLAKEVEN

SEQ ID NO: 21 - DNA, 1650 bp, synthetic construct
  source 1..1650: mol_type = other DNA
atgggccctagcgccttcagctacgtgcgctttagcagcggcaagcaggccaagggcagctctgaacacagacagagagccatgctgggacagtggctggaacagcaccctagcttcacactgagtgatctgcggttcgaggacctgggcagaagcggattcagcggcgagcacctggatcacggcctgggccagctgctggctgctatcgacagcggcgccatcaagagcggagatgtgatcctggtcgaggccgtggacagaatcggcagactggagcctctggaaatgctgcctctgttctccagaatcgtgaaggccggcgtgtccgttatcaccctggaagatggccacgtttacgaccggagctccgtgaacgagacatctctgtttctgctggtggccaaaatccagcaggcccacgagtactctaatagactgtctcgaagaatcaacgcctcttacaccgctcggagagaaaaagctaaagcaggcctgggcatcaagagagagacacctgtgtggctgaccacagacggccaactggtgcctcacgtggcccctcacatcgcccaggcttttcaggactacgccgatggcctgggagagagaaggatttgtagaaagctgcgggagagcggcctggaagaattctccaagaccaacgccaccaccgtgcggagatggctgaagaaccggaccgccattggatattggaacgacatccctgatgtgtaccctcatgtcgtggaccctgctctgttctaccaggtgcagcagcgcctggacgcccctaaggtggacagagccaagcccagcgctcactacctgacaggcctcgtgaagtgcgccgtgtgcggcagaaactacaactacaaacagcggaagcacaccgaccccgctatgctgtgcaccagcagagccagactggccggggaaggctgcagcaatagcaagacataccccgtgatagttctggaccaggtgcggaagctgaccagcctgccgttcctgcaacacgccatggaatccgcctcatctcaggccgacccaagcagccagagactggccgtgatcgacggcgaaatcggcgagctgtccagaaagatcagcgaggccacaaaggccctgctggtgctgggcttcacccctgagatccaggagagcctggaacagctcaagaccgccagagaagccctggaggaagaaagagccaccctgctgctgcctcaggccgagaagctgacaacagctcagctggaggccttcagcaacggcctgctggacgacgagcccatgaagctcaaccacgtgcttcagaccgccggctacagcatggtggtgcaccccgacggctctatcgacgtggatggaaaaagattcgtgtacgagggcgctagccggaaagagaaagtgtacaagctgagactgatcggcgaggataagcagtggagcctgcccatcctgaccccacagatggccacttacaagtccctgttcatggccgctgtgcggctgcctggcgaccccagcgaggaagagctgagacggttcgaggaagccaagcacagcgagcggtcccgtcgtcgtaaggccaacccaaccaagctctccgagaacgccaagaagctcgccaaggaggtcgagaac

SEQ ID NO: 22 - protein, 542 aa, synthetic construct
MGPSAFSYVRFSSGKQAKGSSEHRQRAMLGQWLEQHPSFTLSDLRFEDLGRSGFSGEHLDHGLGQLLAAIDSGAIKSGDVILVEAVDRIGRLEPLEMLPLFSRIVKAGVSVITLEDGHVYDRSSVNETSLFLLVAKIQQAHEYSNRLSRRINASYTARREKAKAGLGIKRETPVWLTTDGQLVPHVAPHIAQAFQDYADGLGERRICRKLRESGLEEFSKTNATTVRRWLKNRTAIGYWNDIPDVYPHVVDPALFYQVQQRLDAPKVDRAKPSAHYLTGLVKCAVCGRNYNYKQRKHTDPAMLCTSRARLAGEGCSNSKTYPVIVLDQVRKLTSLPFLQHAMESASSQADPSSQRLAVIDGEIGELSRKISEATKALLVLGFTPEIQESLEQLKTAREALEEERATLLLPQAEKLTTAQLEAFSNGLLDDEPMKLNHVLQTAGYSMVVHPDGSIDVDGKRFVYEGASRKEKVYKLRLIGEDKQWSLPILTPQMATYKSLFMAAVRLPGDPSEEELRRFEEAKHSERKRPAATKKAGQAKKKK

SEQ ID NO: 23 - DNA, 1626 bp, synthetic construct
  source 1..1626: mol_type = other DNA
atgggccctagcgccttcagctacgtgcgctttagcagcggcaagcaggccaagggcagctctgaacacagacagagagccatgctgggacagtggctggaacagcaccctagcttcacactgagtgatctgcggttcgaggacctgggcagaagcggattcagcggcgagcacctggatcacggcctgggccagctgctggctgctatcgacagcggcgccatcaagagcggagatgtgatcctggtcgaggccgtggacagaatcggcagactggagcctctggaaatgctgcctctgttctccagaatcgtgaaggccggcgtgtccgttatcaccctggaagatggccacgtttacgaccggagctccgtgaacgagacatctctgtttctgctggtggccaaaatccagcaggcccacgagtactctaatagactgtctcgaagaatcaacgcctcttacaccgctcggagagaaaaagctaaagcaggcctgggcatcaagagagagacacctgtgtggctgaccacagacggccaactggtgcctcacgtggcccctcacatcgcccaggcttttcaggactacgccgatggcctgggagagagaaggatttgtagaaagctgcgggagagcggcctggaagaattctccaagaccaacgccaccaccgtgcggagatggctgaagaaccggaccgccattggatattggaacgacatccctgatgtgtaccctcatgtcgtggaccctgctctgttctaccaggtgcagcagcgcctggacgcccctaaggtggacagagccaagcccagcgctcactacctgacaggcctcgtgaagtgcgccgtgtgcggcagaaactacaactacaaacagcggaagcacaccgaccccgctatgctgtgcaccagcagagccagactggccggggaaggctgcagcaatagcaagacataccccgtgatagttctggaccaggtgcggaagctgaccagcctgccgttcctgcaacacgccatggaatccgcctcatctcaggccgacccaagcagccagagactggccgtgatcgacggcgaaatcggcgagctgtccagaaagatcagcgaggccacaaaggccctgctggtgctgggcttcacccctgagatccaggagagcctggaacagctcaagaccgccagagaagccctggaggaagaaagagccaccctgctgctgcctcaggccgagaagctgacaacagctcagctggaggccttcagcaacggcctgctggacgacgagcccatgaagctcaaccacgtgcttcagaccgccggctacagcatggtggtgcaccccgacggctctatcgacgtggatggaaaaagattcgtgtacgagggcgctagccggaaagagaaagtgtacaagctgagactgatcggcgaggataagcagtggagcctgcccatcctgaccccacagatggccacttacaagtccctgttcatggccgctgtgcggctgcctggcgaccccagcgaggaagagctgagacggttcgaggaagccaagcacagcgagcggaaaaggccggcggccacgaaaaaggccggccaggcaaaaaagaaaaag

SEQ ID NO: 24 - protein, 560 aa, synthetic construct
MGPSAFSYVRFSSGKQAKGSSEHRQRAMLGQWLEQHPSFTLSDLRFEDLGRSGFSGEHLDHGLGQLLAAIDSGAIKSGDVILVEAVDRIGRLEPLEMLPLFSRIVKAGVSVITLEDGHVYDRSSVNETSLFLLVAKIQQAHEYSNRLSRRINASYTARREKAKAGLGIKRETPVWLTTDGQLVPHVAPHIAQAFQDYADGLGERRICRKLRESGLEEFSKTNATTVRRWLKNRTAIGYWNDIPDVYPHVVDPALFYQVQQRLDAPKVDRAKPSAHYLTGLVKCAVCGRNYNYKQRKHTDPAMLCTSRARLAGEGCSNSKTYPVIVLDQVRKLTSLPFLQHAMESASSQADPSSQRLAVIDGEIGELSRKISEATKALLVLGFTPEIQESLEQLKTAREALEEERATLLLPQAEKLTTAQLEAFSNGLLDDEPMKLNHVLQTAGYSMVVHPDGSIDVDGKRFVYEGASRKEKVYKLRLIGEDKQWSLPILTPQMATYKSLFMAAVRLPGDPSEEELRRFEEAKHSERKRPAATKKAGQAKKKKGSKRPAATKKAGQAKKKK

SEQ ID NO: 25 - DNA, 1680 bp, synthetic construct
  source 1..1680: mol_type = other DNA
atgggccctagcgccttcagctacgtgcgctttagcagcggcaagcaggccaagggcagctctgaacacagacagagagccatgctgggacagtggctggaacagcaccctagcttcacactgagtgatctgcggttcgaggacctgggcagaagcggattcagcggcgagcacctggatcacggcctgggccagctgctggctgctatcgacagcggcgccatcaagagcggagatgtgatcctggtcgaggccgtggacagaatcggcagactggagcctctggaaatgctgcctctgttctccagaatcgtgaaggccggcgtgtccgttatcaccctggaagatggccacgtttacgaccggagctccgtgaacgagacatctctgtttctgctggtggccaaaatccagcaggcccacgagtactctaatagactgtctcgaagaatcaacgcctcttacaccgctcggagagaaaaagctaaagcaggcctgggcatcaagagagagacacctgtgtggctgaccacagacggccaactggtgcctcacgtggcccctcacatcgcccaggcttttcaggactacgccgatggcctgggagagagaaggatttgtagaaagctgcgggagagcggcctggaagaattctccaagaccaacgccaccaccgtgcggagatggctgaagaaccggaccgccattggatattggaacgacatccctgatgtgtaccctcatgtcgtggaccctgctctgttctaccaggtgcagcagcgcctggacgcccctaaggtggacagagccaagcccagcgctcactacctgacaggcctcgtgaagtgcgccgtgtgcggcagaaactacaactacaaacagcggaagcacaccgaccccgctatgctgtgcaccagcagagccagactggccggggaaggctgcagcaatagcaagacataccccgtgatagttctggaccaggtgcggaagctgaccagcctgccgttcctgcaacacgccatggaatccgcctcatctcaggccgacccaagcagccagagactggccgtgatcgacggcgaaatcggcgagctgtccagaaagatcagcgaggccacaaaggccctgctggtgctgggcttcacccctgagatccaggagagcctggaacagctcaagaccgccagagaagccctggaggaagaaagagccaccctgctgctgcctcaggccgagaagctgacaacagctcagctggaggccttcagcaacggcctgctggacgacgagcccatgaagctcaaccacgtgcttcagaccgccggctacagcatggtggtgcaccccgacggctctatcgacgtggatggaaaaagattcgtgtacgagggcgctagccggaaagagaaagtgtacaagctgagactgatcggcgaggataagcagtggagcctgcccatcctgaccccacagatggccacttacaagtccctgttcatggccgctgtgcggctgcctggcgaccccagcgaggaagagctgagacggttcgaggaagccaagcacagcgagcggaaaaggccggcggccacgaaaaaggccggccaggcaaaaaagaaaaagggatccaaaaggccggcggccacgaaaaaggccggccaggcaaaaaagaaaaag

SEQ ID NO: 26 - DNA, 104 bp, unidentified
  source 1..104: mol_type = other DNA
ccggtttcccttcgcacccgcaccgcggcttcgagaccgtgacctacatgctcgaagggcgtatgcgccacgaagaccacctcggcaatcgcggcctgctcaag

SEQ ID NO: 27 - DNA, 65 bp, unidentified
  source 1..65: mol_type = other DNA
gcaccgcggcttcgagaccgtgacctacatgctcgaagggcgtatgcgccacgaagaccacctcg

SEQ ID NO: 28 - DNA, 40 bp, unidentified
  source 1..40: mol_type = other DNA
gaccgtgacctacatgctcgaagggcgtatgcgccacgaa

SEQ ID NO: 29 - DNA, 33 bp, unidentified
  source 1..33: mol_type = other DNA
ccgtgacctacatgctcgaagggcgtatgcgcc

SEQ ID NO: 30 - DNA, 104 bp, unidentified
  source 1..104: mol_type = other DNA
gtaacgctcttcgagaaagcagattctcatatccatcttgagtcttctttctcgcaagacaacacgaaatagacacagtctcttccctagctgtacactgagcc

SEQ ID NO: 31 - DNA, 33 bp, synthetic construct
  source 1..33: mol_type = other DNA
ccgtgacctacatgcnngaagggcgtatgcgcc

SEQ ID NO: 32 - DNA, 40 bp, synthetic construct
  source 1..40: mol_type = other DNA
gaccgtgacctacatgcnngaagggcgtatgcgccacgaa

SEQ ID NO: 33 - DNA, 65 bp, synthetic construct
  source 1..65: mol_type = other DNA
gcaccgcggcttcgagaccgtgacctacatgcnngaagggcgtatgcgccacgaagaccacctcg

SEQ ID NO: 34 - DNA, 104 bp, synthetic construct
  source 1..104: mol_type = other DNA
ccggtttcccttcgcacccgcaccgcggcttcgagaccgtgacctacatgcnngaagggcgtatgcgccacgaagaccacctcggcaatcgcggcctgctcaag

SEQ ID NO: 35 - DNA, 33 bp, synthetic construct
  source 1..33: mol_type = other DNA
ccgtgacctacatgcaggaagggcgtatgcgcc

SEQ ID NO: 36 - DNA, 33 bp, synthetic construct
  source 1..33: mol_type = other DNA
ccgtgacctacatgcacgaagggcgtatgcgcc

SEQ ID NO: 37 - DNA, 33 bp, synthetic construct
  source 1..33: mol_type = other DNA
ccgtgacctacatgcatgaagggcgtatgcgcc

SEQ ID NO: 38 - DNA, 33 bp, synthetic construct
  source 1..33: mol_type = other DNA
ccgtgacctacatgcaagaagggcgtatgcgcc

SEQ ID NO: 39 - DNA, 33 bp, synthetic construct
  source 1..33: mol_type = other DNA
ccgtgacctacatgctggaagggcgtatgcgcc

SEQ ID NO: 40 - DNA, 33 bp, synthetic construct; identical to SEQ ID NO: 29
  source 1..33: mol_type = other DNA

SEQ ID NO: 41 - DNA, 33 bp, synthetic construct
  source 1..33: mol_type = other DNA
ccgtgacctacatgcttgaagggcgtatgcgcc

SEQ ID NO: 42 - DNA, 33 bp, synthetic construct
  source 1..33: mol_type = other DNA
ccgtgacctacatgctagaagggcgtatgcgcc

SEQ ID NO: 43 - DNA, 33 bp, synthetic construct
  source 1..33: mol_type = other DNA
ccgtgacctacatgccggaagggcgtatgcgcc

SEQ ID NO: 44 - DNA, 33 bp, synthetic construct
  source 1..33: mol_type = other DNA
ccgtgacctacatgcccgaagggcgtatgcgcc

SEQ ID NO: 45 - DNA, 33 bp, synthetic construct
  source 1..33: mol_type = other DNA
ccgtgacctacatgcctgaagggcgtatgcgcc

SEQ ID NO: 46 - DNA, 33 bp, synthetic construct
  source 1..33: mol_type = other DNA
ccgtgacctacatgccagaagggcgtatgcgcc

SEQ ID NO: 47 - DNA, 33 bp, synthetic construct
  source 1..33: mol_type = other DNA
ccgtgacctacatgcgggaagggcgtatgcgcc

SEQ ID NO: 48 - DNA, 33 bp, synthetic construct
  source 1..33: mol_type = other DNA
ccgtgacctacatgcgcgaagggcgtatgcgcc

SEQ ID NO: 49 - DNA, 33 bp, synthetic construct
  source 1..33: mol_type = other DNA
ccgtgacctacatgcgtgaagggcgtatgcgcc

SEQ ID NO: 50 - DNA, 33 bp, synthetic construct
  source 1..33: mol_type = other DNA
ccgtgacctacatgcgagaagggcgtatgcgcc

SEQ ID NO: 51 - DNA, 36 bp, synthetic construct
  source 1..36: mol_type = other DNA
atcttgagtcttctttcnngcaagacaacacgaaat

SEQ ID NO: 52 - DNA, 104 bp, synthetic construct
  source 1..104: mol_type = other DNA
gtaacgctcttcgagaaagcagattctcatatccatcttgagtcttctttcnngcaagacaacacgaaatagacacagtctcttccctagctgtacactgagcc

SEQ ID NO: 53 - DNA, 36 bp, synthetic construct
  source 1..36: mol_type = other DNA
atcttgagtcttctttcaggcaagacaacacgaaat

SEQ ID NO: 54 - DNA, 36 bp, synthetic construct
  source 1..36: mol_type = other DNA
atcttgagtcttctttcacgcaagacaacacgaaat

SEQ ID NO: 55 - DNA, 36 bp, synthetic construct
  source 1..36: mol_type = other DNA
atcttgagtcttctttcatgcaagacaacacgaaat

SEQ ID NO: 56 - DNA, 36 bp, synthetic construct
  source 1..36: mol_type = other DNA
atcttgagtcttctttcaagcaagacaacacgaaat

SEQ ID NO: 57 - DNA, 36 bp, synthetic construct
  source 1..36: mol_type = other DNA
atcttgagtcttctttctggcaagacaacacgaaat

SEQ ID NO: 58 - DNA, 36 bp, synthetic construct
  source 1..36: mol_type = other DNA
atcttgagtcttctttctcgcaagacaacacgaaat

SEQ ID NO: 59 - DNA, 36 bp, synthetic construct
  source 1..36: mol_type = other DNA
atcttgagtcttctttcttgcaagacaacacgaaat

SEQ ID NO: 60 - DNA, 36 bp, synthetic construct
  source 1..36: mol_type = other DNA
atcttgagtcttctttctagcaagacaacacgaaat

SEQ ID NO: 61 - DNA, 36 bp, synthetic construct
  source 1..36: mol_type = other DNA
atcttgagtcttctttccggcaagacaacacgaaat

SEQ ID NO: 62 - DNA, 36 bp, synthetic construct
  source 1..36: mol_type = other DNA
atcttgagtcttctttcccgcaagacaacacgaaat

SEQ ID NO: 63 - DNA, 36 bp, synthetic construct
  source 1..36: mol_type = other DNA
atcttgagtcttctttcctgcaagacaacacgaaat

SEQ ID NO: 64 - DNA, 36 bp, synthetic construct
  source 1..36: mol_type = other DNA
atcttgagtcttctttccagcaagacaacacgaaat

SEQ ID NO: 65 - DNA, 36 bp, synthetic construct
  source 1..36: mol_type = other DNA
atcttgagtcttctttcgggcaagacaacacgaaat

SEQ ID NO: 66 - DNA, 36 bp, synthetic construct
  source 1..36: mol_type = other DNA
atcttgagtcttctttcgcgcaagacaacacgaaat

SEQ ID NO: 67 - DNA, 36 bp, synthetic construct
  source 1..36: mol_type = other DNA
atcttgagtcttctttcgtgcaagacaacacgaaat

SEQ ID NO: 68 - DNA, 36 bp, synthetic construct
  source 1..36: mol_type = other DNA
atcttgagtcttctttcgagcaagacaacacgaaat

SEQ ID NO: 69 - DNA, 82 bp, unidentified
  source 1..82: mol_type = other DNA
cgagaaagcagattctcatatccatcttgagtcttctttctcgcaagacaacacgaaatagacacagtctcttccctagctg

SEQ ID NO: 70 - DNA, 52 bp, unidentified
  source 1..52: mol_type = other DNA
tcatatccatcttgagtcttctttctcgcaagacaacacgaaatagacacag

SEQ ID NO: 71 - DNA, 36 bp, unidentified; identical to SEQ ID NO: 58
  source 1..36: mol_type = other DNA

SEQ ID NO: 72 - DNA, 52 bp, synthetic construct
  source 1..52: mol_type = other DNA
tcatatccatcttgagtcttctttcnngcaagacaacacgaaatagacacag

SEQ ID NO: 73 - DNA, 82 bp, synthetic construct
  source 1..82: mol_type = other DNA
cgagaaagcagattctcatatccatcttgagtcttctttcnngcaagacaacacgaaatagacacagtctcttccctagctg

SEQ ID NO: 74 - DNA, 1578 bp, unidentified
  source 1..1578: mol_type = other DNA
atgggccctagcgccttcagctacgtgcgctttagcagcggcaagcaggccaagggcagctctgaacacagacagagagccatgctgggacagtggctggaacagcaccctagcttcacactgagtgatctgcggttcgaggacctgggcagaagcggattcagcggcgagcacctggatcacggcctgggccagctgctggctgctatcgacagcggcgccatcaagagcggagatgtgatcctggtcgaggccgtggacagaatcggcagactggagcctctggaaatgctgcctctgttctccagaatcgtgaaggccggcgtgtccgttatcaccctggaagatggccacgtttacgaccggagctccgtgaacgagacatctctgtttctgctggtggccaaaatccagcaggcccacgagtactctaatagactgtctcgaagaatcaacgcctcttacaccgctcggagagaaaaagctaaagcaggcctgggcatcaagagagagacacctgtgtggctgaccacagacggccaactggtgcctcacgtggcccctcacatcgcccaggcttttcaggactacgccgatggcctgggagagagaaggatttgtagaaagctgcgggagagcggcctggaagaattctccaagaccaacgccaccaccgtgcggagatggctgaagaaccggaccgccattggatattggaacgacatccctgatgtgtaccctcatgtcgtggaccctgctctgttctaccaggtgcagcagcgcctggacgcccctaaggtggacagagccaagcccagcgctcactacctgacaggcctcgtgaagtgcgccgtgtgcggcagaaactacaactacaaacagcggaagcacaccgaccccgctatgctgtgcaccagcagagccagactggccggggaaggctgcagcaatagcaagacataccccgtgatagttctggaccaggtgcggaagctgaccagcctgccgttcctgcaacacgccatggaatccgcctcatctcaggccgacccaagcagccagagactggccgtgatcgacggcgaaatcggcgagctgtccagaaagatcagcgaggccacaaaggccctgctggtgctgggcttcacccctgagatccaggagagcctggaacagctcaagaccgccagagaagccctggaggaagaaagagccaccctgctgctgcctcaggccgagaagctgacaacagctcagctggaggccttcagcaacggcctgctggacgacgagcccatgaagctcaaccacgtgcttcagaccgccggctacagcatggtggtgcaccccgacggctctatcgacgtggatggaaaaagattcgtgtacgagggcgctagccggaaagagaaagtgtacaagctgagactgatcggcgaggataagcagtggagcctgcccatcctgaccccacagatggccacttacaagtccctgttcatggccgctgtgcggctgcctggcgaccccagcgaggaagagctgagacggttcgaggaagccaagcacagcgagcgg